European Patent Specification EP 3 845 557 B1, published August 2, 2023. Title: Method to Treat Cancer with Engineered T-Cells. Applicant: Lentigen Technology, Inc. Application EP16808492.9. The sequence listing filed with the application follows.

SEQUENCE LISTING (32 sequences)

SEQ ID NO: 1-4 - skipped (4 entries)

SEQ ID NO: 5 - DNA, 66 bp, Artificial Sequence
  leader/signal peptide
atgctgctgctggtgaccagcctgctgctgtgcgaactgccgcatccggcgtttctgctgattccg

SEQ ID NO: 6 - protein, 22 aa, Artificial Sequence
  leader/signal peptide
MLLLVTSLLLCELPHPAFLLIP

SEQ ID NO: 7-10 - skipped (4 entries)

SEQ ID NO: 11 - DNA, 72 bp, Artificial Sequence
  CD8 transmembrane domain
atctacatctgggcgcccttggccgggacttgtggggtccttctcctgtcactggttatcaccctttactgc

SEQ ID NO: 12 - protein, 22 aa, Artificial Sequence
  CD8 transmembrane domain
IWAPLAGTCGVLLLSLVITLYC

SEQ ID NO: 13 - DNA, 135 bp, Artificial Sequence
  CD8 hinge domain
accacgacgccagcgccgcgaccaccaacaccggcgcccaccatcgcgtcgcagcccctgtccctgcgcccagaggcgtgccggccagcggcggggggcgcagtgcacacgagggggctggacttcgcctgtgat

SEQ ID NO: 14 - protein, 47 aa, Artificial Sequence
  CD8 hinge domain
TTTPAPRPPTPAPTIASQPLSLRPEACRPAAGGAVHTRGLDFACDIY

SEQ ID NO: 15 - protein, 42 aa, Artificial Sequence
  amino acid residues 118-178 of CD8.alpha. hinge region
KRGRKKLLYIFKQPFMRPVQTTQEEDGCSCRFPEEEEGGCEL

SEQ ID NO: 16 - protein, 106 aa, Homo sapiens
  MISC_FEATURE: IgGCL region
GQPKAAPSVTLFPPSSEELQANKATLVCLISDFYPGAVTVAWKADSSPVKAGVETTTPSKQSNNKYAASSYLSLTPEQWKSHRSYSCQVTHEGSTVEKTVAPTECS

SEQ ID NO: 17 - DNA, 126 bp, Artificial Sequence
  signaling domain of 4-lBB
aaacggggcagaaagaaactcctgtatatattcaaacaaccatttatgagaccagtacaaactactcaagaggaagatggctgtagctgccgatttccagaagaagaagaaggaggatgtgaactg

SEQ ID NO: 18 - protein, 42 aa, Artificial Sequence; identical to SEQ ID NO: 15
  signaling domain of 4-lBB

SEQ ID NO: 19 - DNA, 336 bp, Artificial Sequence
  signaling domain of CD3-zeta
agagtgaagttcagcaggagcgcagacgcccccgcgtacaagcagggccagaaccagctctataacgagctcaatctaggacgaagagaggagtacgatgttttggacaagagacgtggccgggaccctgagatggggggaaagccgagaaggaagaaccctcaggaaggcctgtacaatgaactgcagaaagataagatggcggaggcctacagtgagattgggatgaaaggcgagcgccggaggggcaaggggcacgatggcctttaccagggtctcagtacagccaccaaggacacctacgacgcccttcacatgcaggccctgccccctcgc

SEQ ID NO: 20 - protein, 112 aa, Artificial Sequence
  CD3zeta
RVKFSRSADAPAYKQGQNQLYNELNLGRREEYDVLDKRRGRDPEMGGKPRRKNPQEGLYNELQKDKMAEAYSEIGMKGERRRGKGHDGLYQGLSTATKDTYDALHMQALPPR

SEQ ID NO: 21 - DNA, 1467 bp, Artificial Sequence
  SPCD19binder-CD8link-CD4tm-signals LTG 1562
atgctgctgctggtgaccagcctgctgctgtgcgaactgccgcatccggcgtttctgctgattccggatattcagatgacccagaccaccagcagcctgagcgcgagcctgggcgatcgcgtgaccattagctgccgcgcgagccaggatattagcaaatatctgaactggtatcagcagaaaccggatggcaccgtgaaactgctgatttatcataccagccgcctgcatagcggcgtgccgagccgctttagcggcagcggcagcggcaccgattatagcctgaccattagcaacctggaacaggaagatattgcgacctatttttgccagcagggcaacaccctgccgtatacctttggcggcggcaccaaactggaaattaccggcggcggcggcagcggcggcggcggcagcggcggcggcggcagcgaagtgaaactgcaggaaagcggcccgggcctggtggcgccgagccagagcctgagcgtgacctgcaccgtgagcggcgtgagcctgccggattatggcgtgagctggattcgccagccgccgcgcaaaggcctggaatggctgggcgtgatttggggcagcgaaaccacctattataacagcgcgctgaaaagccgcctgaccattattaaagataacagcaaaagccaggtgtttctgaaaatgaacagcctgcagaccgatgataccgcgatttattattgcgcgaaacattattattatggcggcagctatgcgatggattattggggccagggcaccagcgtgaccgtgagcagcgcggcggcgccggcgccgcgcccgccgaccccggcgccgaccattgcgagccagccgctgagcctgcgcccggaagcgtgccgcccggcggcgggcggcgcggtgcatacccgcggcctggattttgtgcagccgatggcgctgattgtgctgggcggcgtggcgggcctgctgctgtttattggcctgggcatttttttttgcgtgcgctgccgcccgcgccgcaaaaaactgctgtatatttttaaacagccgtttatgcgcccggtgcagaccacccaggaagaagatggctgcagctgccgctttccggaagaagaagaaggcggctgcgaactgcgcgtgaaatttagccgcagcgcggatgcgccggcgtatcagcagggccagaaccagctgtataacgaactgaacctgggccgccgcgaagaatatgatgtgctggataaacgccgcggccgcgatccggaaatgggcggcaaaccgcgccgcaaaaacccgcaggaaggcctgtataacgaactgcagaaagataaaatggcggaagcgtatagcgaaattggcatgaaaggcgaacgccgccgcggcaaaggccatgatggcctgtatcagggcctgagcaccgcgaccaaagatacctatgatgcgctgcatatgcaggcgctgccgccgcgc

SEQ ID NO: 22 - protein, 485 aa, Artificial Sequence
  SP-CD19binder-CD8link-CD4tm-signals LTG1562
MLLLVTSLLLCELPHPAFLLIPDIQMTQTTSSLSASLGDRVTISCRASQDISKYLNWYQQKPDGTVKLLIYHTSRLHSGVPSRFSGSGSGTDYSLTISNLEQEDIATYFCQQGNTLPYTFGGGTKLEITGGGGSGGGGSGGGGSEVKLQESGPGLVAPSQSLSVTCTVSGVSLPDYGVSWIRQPPRKGLEWLGVIWGSETTYYNSALKSRLTIIKDNSKSQVFLKMNSLQTDDTAIYYCAKHYYYGGSYAMDYWGQGTSVTVSSAAAPAPRPPTPAPTIASQPLSLRPEACRPAAGGAVHTRGLDFVQPMALIVLGGVAGLLLFIGLGIFFCVRCRPRRKKLLYIFKQPFMRPVQTTQEEDGCSCRFPEEEEGGCELRVKFSRSADAPAYQQGQNQLYNELNLGRREEYDVLDKRRGRDPEMGGKPRRKNPQEGNELQKDKMAEAYSEIGMKGERRRGKGHDGQGLSTATKDTYDALHMQALPPR

SEQ ID NO: 23-26 - skipped (4 entries)

SEQ ID NO: 27 - DNA, 726 bp, Artificial Sequence
  anti-CD19 scvf
gacatccagatgacacagactacatcctccctgtctgcctctctgggagacagagtcaccatcagttgcagggcaagtcaggacattagtaaatatttaaattggtatcagcagaaaccagatggaactgttaaactcctgatctaccatacatcaagattacactcaggagtcccatcaaggttcagtggcagtgggtctggaacagattattctctcaccattagcaacctggagcaagaagatattgccacttacttttgccaacagggtaatacgcttccgtacacgttcggaggggggaccaagctggagatcacaggtggcggtggctcgggcggtggtgggtcgggtggcggcggatctgaggtgaaactgcaggagtcaggacctggcctggtggcgccctcacagagcctgtccgtcacatgcactgtctcaggggtctcattacccgactatggtgtaagctggattcgccagcctccacgaaagggtctggagtggctgggagtaatatggggtagtgaaaccacatactataattcagctctcaaatccagactgaccatcatcaaggacaactccaagagccaagttttcttaaaaatgaacagtctgcaaactgatgacacagccatttactactgtgccaaacattattactacggtggtagctatgctatggactactggggccaaggaacctcagtcaccgtctcctca

SEQ ID NO: 28 - protein, 242 aa, Artificial Sequence
  anti-CD19 scvf
DIQMTQTTSSLSASLGDRVTISCRASQDISKYLNWYQQKPDGTVKLLIYHTSRLHSGVPSRFSGSGSGTDYSLTISNLEQEDIATYFCQQGNTLPYTFGGGTKLEITGGGGSGGGGSGGGGSEVKLQESGPGLVAPSQSLSVTCTVSGVSLPDYGVSWIRQPPRKGLEWLGVIWGSETTYYNSALKSRLTIIKDNSKSQVFLKMNSLQTDDTAIYYCAKHYYYGGSYAMDYWGQGTSVTVSS

SEQ ID NO: 29 - DNA, 1485 bp, Artificial Sequence
  SP-CD19binder-CD8link-CD8tm-signaling LTG1494
atgctgctgctggtgaccagcctgctgctgtgcgaactgccgcatccggcgtttctgctgattccggataccgatattcagatgacccagaccaccagcagcctgagcgcgagcctgggcgatcgcgtgaccattagctgccgcgcgagccaggatattagcaaatatctgaactggtatcagcagaaaccggatggcaccgtgaaactgctgatttatcataccagccgcctgcatagcggcgtgccgagccgctttagcggcagcggcagcggcaccgattatagcctgaccattagcaacctggaacaggaagatattgcgacctatttttgccagcagggcaacaccctgccgtatacctttggcggcggcaccaaactggaaattaccggcagcaccagcggcagcggcaaaccgggcagcggcgaaggcagcaccaaaggcgaagtgaaactgcaggaaagcggcccgggcctggtggcgccgagccagagcctgagcgtgacctgcaccgtgagcggcgtgagcctgccggattatggcgtgagctggattcgccagccgccgcgcaaaggcctggaatggctgggcgtgatttggggcagcgaaaccacctattataacagcgcgctgaaaagccgcctgaccattattaaagataacagcaaaagccaggtgtttctgaaaatgaacagcctgcagaccgatgataccgcgatttattattgcgcgaaacattattattatggcggcagctatgcgatggattattggggccagggcaccagcgtgaccgtgagcagcgcggcggcgaccaccaccccggcgccgcgcccgccgaccccggcgccgaccattgcgagccagccgctgagcctgcgcccggaagcgtgccgcccggcggcgggcggcgcggtgcatacccgcggcctggattttgcgtgcgatatttatatttgggcgccgctggcgggcacctgcggcgtgctgctgctgagcctggtgattaccctgtattgcaaacgcggccgcaaaaaactgctgtatatttttaaacagccgtttatgcgcccggtgcagaccacccaggaagaagatggctgcagctgccgctttccggaagaagaagaaggcggctgcgaactgcgcgtgaaatttagccgcagcgcggatgcgccggcgtatcagcagggccagaaccagctgtataacgaactgaacctgggccgccgcgaagaatatgatgtgctggataaacgccgcggccgcgatccggaaatgggcggcaaaccgcgccgcaaaaacccgcaggaaggcctgtataacgaactgcagaaagataaaatggcggaagcgtatagcgaaattggcatgaaaggcgaacgccgccgcggcaaaggccatgatggcctgtatcagggcctgagcaccgcgaccaaagatacctatgatgcgctgcatatgcaggcgctgccgccgcgc

SEQ ID NO: 30 - protein, 491 aa, Artificial Sequence
  SP-CD19binder-CD8link-CD8tm-signaling LTG1494
MLLLVTSLLLCELPHPAFLLIPDTDIQMTQTTSSLSASLGDRVTISCRASQDISKYLNWYQQKPDGTVKLLIYHTSRLHSGVPSRFSGSGSGTDYSLTISNLEQEDIATYFCQQGNTLPYTFGGGTKLEITGSTSGSGKPGSGEGSTKGEVKLQESGPGLVAPSQSLSVTCTVSGVSLPDYGVSWIRQPPRKGLEWLGVIWGSETTYYNSALKSRLTIIKDNSKSQVFLKMNSLQTDDTAIYYCAKHYYYGGSYAMDYWGQGTSVTVSSAAATTTPAPRPPTPAPTIASQPLSLRPEACRPAAGGAVHTRGLDFACDIYIWAPLAGTCGVLLLSLVITLYCKRGRKKLLYIFKQPFMRPVQTTQEEDGCSCRFPEEEEGGCELRVKFSRSADAPAYQQGQNQLYNELNLGRREEYDVLDKRRGRDPEMGGKPRRKNPQEGNELQKDKMAEAYSEIGMKGERRRGKGHDGQGLSTATKDTYDALHMQALPPR

SEQ ID NO: 31 - DNA, 1470 bp, Artificial Sequence
  SP-CD19binder-CD8link-CD8tm-signals (LTI re-engineered) (CTG 1538)
atgctgctgctggtgaccagcctgctgctgtgcgaactgccgcatccggcgtttctgctgattccggatattcagatgacccagaccaccagcagcctgagcgcgagcctgggcgatcgcgtgaccattagctgccgcgcgagccaggatattagcaaatatctgaactggtatcagcagaaaccggatggcaccgtgaaactgctgatttatcataccagccgcctgcatagcggcgtgccgagccgctttagcggcagcggcagcggcaccgattatagcctgaccattagcaacctggaacaggaagatattgcgacctatttttgccagcagggcaacaccctgccgtatacctttggcggcggcaccaaactggaaattaccggcggcggcggcagcggcggcggcggcagcggcggcggcggcagcgaagtgaaactgcaggaaagcggcccgggcctggtggcgccgagccagagcctgagcgtgacctgcaccgtgagcggcgtgagcctgccggattatggcgtgagctggattcgccagccgccgcgcaaaggcctggaatggctgggcgtgatttggggcagcgaaaccacctattataacagcgcgctgaaaagccgcctgaccattattaaagataacagcaaaagccaggtgtttctgaaaatgaacagcctgcagaccgatgataccgcgatttattattgcgcgaaacattattattatggcggcagctatgcgatggattattggggccagggcaccagcgtgaccgtgagcagcgcggcggcgaccaccaccccggcgccgcgcccgccgaccccggcgccgaccattgcgagccagccgctgagcctgcgcccggaagcgtgccgcccggcggcgggcggcgcggtgcatacccgcggcctggattttgcgtgcgatatttatatttgggcgccgctggcgggcacctgcggcgtgctgctgctgagcctggtgattaccctgtattgcaaacgcggccgcaaaaaactgctgtatatttttaaacagccgtttatgcgcccggtgcagaccacccaggaagaagatggctgcagctgccgctttccggaagaagaagaaggcggctgcgaactgcgcgtgaaatttagccgcagcgcggatgcgccggcgtatcagcagggccagaaccagctgtataacgaactgaacctgggccgccgcgaagaatatgatgtgctggataaacgccgcggccgcgatccggaaatgggcggcaaaccgcgccgcaaaaacccgcaggaaggcctgtataacgaactgcagaaagataaaatggcggaagcgtatagcgaaattggcatgaaaggcgaacgccgccgcggcaaaggccatgatggcctgtatcagggcctgagcaccgcgaccaaagatacctatgatgcgctgcatatgcaggcgctgccgccgcgc

SEQ ID NO: 32 - protein, 486 aa, Artificial Sequence
  SP-CD19binder-CD8link-CD8tm-signals (LTI re-engineered) (LTG 1538)
MLLLVTSLLLCELPHPAFLLIPDIQMTQTTSSLSASLGDRVTISCRASQDISKYLNWYQQKPDGTVKLLIYHTSRLHSGVPSRFSGSGSGTDYSLTISNLEQEDIATYFCQQGNTLPYTFGGGTKLEITGGGGSGGGGSGGGGSEVKLQESGPGLVAPSQSLSVTCTVSGVSLPDYGVSWIRQPPRKGLEWLGVIWGSETTYYNSALKSRLTIIKDNSKSQVFLKMNSLQTDDTAIYYCAKHYYYGGSYAMDYWGQGTSVTVSSAAATTTPAPRPPTPAPTIASQPLSLRPEACRPAAGGAVHTRGLDFACDIYIWAPLAGTCGVLLLSLVITLYCKRGRKKLLYIFKQPFMRPVQTTQEEDGCSCRFPEEEEGGCELRVKFSRSADAPAYQQGQNQLYNELNLGRREEYDVLDKRRGRDPEMGGKPRRKNPQEGNELQKDKMAEAYSEIGMKGERRRGKGHDGQGLSTATKDTYDALHMQALPPR